European Patent Specification EP 3 491 915 B1, published May 31, 2023. Title: Method for removing genetic linkage in a plant. Applicant: Keygene N.V. The sequence listing filed with the application follows.

SEQUENCE LISTING (12 sequences)

SEQ ID NO: 1 - DNA, 25 bp, Artificial Sequence
  primer ALS2
tgggaatggtggttcagtgggagga

SEQ ID NO: 2 - DNA, 26 bp, Artificial Sequence
  primer ALS2
ggtggttcagtgggaggatcgattct

SEQ ID NO: 3 - DNA, 25 bp, Artificial Sequence
  primer ALS2
cgtagctcccggaccagatgtagca

SEQ ID NO: 4 - DNA, 29 bp, Artificial Sequence
  primer ALS2
atgtagcaatacaaacaccagggaaccca

SEQ ID NO: 5 - DNA, 18 bp, Artificial Sequence
  additional primer
tcaccccttcaccttacc

SEQ ID NO: 6 - DNA, 20 bp, Artificial Sequence
  additional primer 2
ccttcacatttaaccaaagc

SEQ ID NO: 7 - DNA, 19 bp, Artificial Sequence
  primers ALS2
gaaagggaaggggttaagg

SEQ ID NO: 8 - DNA, 18 bp, Artificial Sequence
  primer als2
cttcagtagagcccttgc

SEQ ID NO: 9 - DNA, 18 bp, Artificial Sequence
  primer pcr
cttgtggaggcacttgaa

SEQ ID NO: 10 - DNA, 20 bp, Artificial Sequence
  more primers
ccggaccagatgtagcaata

SEQ ID NO: 11 - DNA, 22 bp, Artificial Sequence
  primer
cttccacccttcttcccaaatc

SEQ ID NO: 12 - DNA, 20 bp, Artificial Sequence
  primer
tgccaactcctgcacattca